European Patent Application EP 4 678 653 A1, published January 14, 2026. Title: muNS FUSION PROTEIN CAPABLE OF FORMING MICROSPHERES AND USES THEREOF. Applicant: UNIVERSIDADE DE SANTIAGO DE COMPOSTELA. The sequence listing filed with the application follows.

SEQUENCE LISTING (37 sequences)

SEQ ID NO: 1 - protein, 188 aa, Avian orthoreovirus
PAALLSKIADLQRANRELSLKLVDVQPAREDHLLAYLNEHVCVNAKDHEKGLLARCNVSGDSISSILGQRMKNRERFETRLRHEASAEWEPRVEALNQELAKARVEQQDMMTQSLQYLNERDELLQEVDELKRELTTLRSANVRLNADNHRMSRATRVGDAFVSDVEPLPSGIPGESKPSMEELVDDL

SEQ ID NO: 2 - protein, 204 aa, Mammalian orthoreovirus
VALQPLLSQLRELSSEVTRLQMELSRAQSLNAQLEADVKSAQSCSLDMYLRHHTCINGHAKEDELLDAVRVAPDVRREIMEKRSEVRQGWCERISKEAAAKCQTVIDDLTLMNGKQAQEITELRDSAEKYEKQIAELVSTITQNQITYQQELQALVAKNVELDALNQRQAKSLRITPSLLSATPIDSADGVADLIDFSVPTDEL

SEQ ID NO: 3 - protein, 635 aa, Avian orthoreovirus
MASTKWGDKPMSVSMSHDGSSIRSAASQFLSGPLFHSTPIPPQRKTVLLKFMIGDELVTVQGALAPFDEYWYDNQPLLAQAVEMLASADRLRQFEHYEKFLLKKGHQITEIMNRLRLFFTDVLKVKMEADALPALAQYLMVGTLEAVSTADSPDACVPVTSKILAKQQTIAKSPGRLDEEEYNVIRSRFLTHEVFDLTSDLPGVQPFMDMYYATVPRADSTGWCVYRRKGLLIHAPDEQFSDLTIFSTRLTASRELQLVAGDVAVACFDLMDVSDIAPSHHASVQEERTLGTSRYSNVTANDHPLVFFSPSALRWAIDHACTDSLVSTRNIRVCVGIDPLVTRWTRDGVQEAAILMDDKLPSAGRARMALRTLLLARRSPMTSFLLGALKQSGGQLMEHYRCDAANRYGSPTVPVSHSPPCSKCPELKEQITKLSSSPLPKIDSNVGPAALLSKIADLQRANRELSLKLVDVQPAREDHLLAYLNEHVCVNAKDHEKGLLSRCNVSGDSISSILGQRVKNRERFETRLRHEASAEWEPRVEALNQELAKARVEQQDMMTQSLQYLNERDELLHEVDELKRELTTLRSANVRLNADNHRMSRATRVGDAFVSDVEPLPSGIPGESKPSMEELVDDL

SEQ ID NO: 4 - protein, 721 aa, Mammalian orthoreovirus
MASFKGFSANTVPVSKAKRDISSLAATPGLRSQSFTPSVDMSQSREFLTKAIEQGSMSIPYQHVNVPKVDRKVVSLVVRPFSSGAFSISGVISPAHAYLLECLPQLEQAMAFVASPESFQASDVAKRFAIKPGMSLQDAITAFINFVSAMLKMTVTRQNFDVIVAEIERLASTSVSVRTKEAKVADEELMLFGLDHRGPQQLDVSDAKGIMKAADIQTTHDVHLAPGVGNIDPEIYNEGRFMFMQHKPLAADQSYFTLETADYFKIYPTYDEHDGRMADQKQSGLILCTKDEVLAEQTIFKLDAPDDKTVHLLDRDDDHVVARFTKVFIEDVAPGHHAAQRSGQRSVLDDLYANTQVISITSAALKWVVKHGVSDGIVNRKNVKVCVGFDPLYTLSTHNGVSLCALLMDEKLSVLNSACRMTLRSLMKTGRDVDAHRAFQRVLSQGYTSLMCYYHPSRKLAYGEVLFLERSNDVTDGIKLQLDASRQCHECPVLQQKVVELEKQIIMQKSIQSDPTPVALQPLLSQLRELSSEVTRLQMELSRAQSLNAQLEADVKSAQSCSLDMYLRHHTCINGHAKEDELLDAVRVAPDVRREIMEKRSEVRQGWCERISKEAAAKCQTVIDDLTLMNGKQAQEITELRDSAEKYEKQIAELVSTITQNQITYQQELQALVAKNVELDALNQRQAKSLRITPSLLSATPIDSADGVADLIDFSVPTDEL

SEQ ID NO: 5 - protein, 5 aa, synthetic construct
  source 1..5: note = enterokinase cleavage site
DDDDK

SEQ ID NO: 6 - protein, 5 aa, Synthetic construct
  source 1..5: note = Xa factor cleavage site
IEDGR

SEQ ID NO: 7 - protein, 6 aa, synthetic construct
  source 1..6: note = thrombin cleavage site
LVPRGS

SEQ ID NO: 8 - protein, 7 aa, synthetic construct
  source 1..7: note = TEV protease cleavage site
ENLYFQG

SEQ ID NO: 9 - protein, 8 aa, synthetic construct
  source 1..8: note = protease PreScission cleavage site
LEVLFQGP

SEQ ID NO: 10 - protein, 20 aa, synthetic construct
  source 1..20: note = Signal peptide
MGWSLILLFLVAVATGVHSQ

SEQ ID NO: 11 - protein, 29 aa, synthetic construct
  source 1..29: note = Signal peptide
MMSFVSLLLVGILFWATEAEQLTKCEVFQ

SEQ ID NO: 12 - protein, 25 aa, synthetic construct
  source 1..25: note = human PTH1R
MGTARIAPGLALLLCCPVLSSAYAL

SEQ ID NO: 13 - protein, 25 aa, synthetic construct
  source 1..25: note = human cytochrome c oxidase VIII mitochondrial signal peptide
MSVLTPLLLRGLTGSARRLPVPRAK

SEQ ID NO: 14 - protein, 20 aa, synthetic construct
  source 1..20: note = human mGluR5 signal peptide
MVLLLILSVLLLKEDVRGSA

SEQ ID NO: 15 - protein, 38 aa, synthetic construct
  source 1..38: note = human GABAB2R signal peptide
MASPRSSGQPGPPPPPPPPPARLLLLLLLPLLLPLAPG

SEQ ID NO: 16 - protein, 17 aa, synthetic construct
  source 1..17: note = human calreticulin signal peptide
MLLSVPLLLGLLGLAVA

SEQ ID NO: 17 - protein, 31 aa, synthetic construct
  source 1..31: note = Human IgGamma2b heavy chain signal peptide
MGWSCIILFLVATATGKGLTVAGLRSGHIYG

SEQ ID NO: 18 - protein, 188 aa, synthetic construct
  source 1..188: note = avian muNS-Mi N57S
PAVLLSKIADLQRANRELSLKLVDVQPAREDHLLAYLNEHVCVNAKDHEKGLLARCSVSGDSISSILGQRMKNRERFETRLRHEASAEWEPRVEALNQELAKARVEQQDMMTQSLQYLNERDELLQEVDELKRELTTLRSANVRLNADNHRMSRATRVGDAFVSDVEPLPSGIPGESKPSMEELVDDL

SEQ ID NO: 19 - protein, 204 aa, synthetic construct
  source 1..204: note = mammalian muNS-Mi N57S
VALQPLLSQLRELSSEVTRLQMELSRAQSLNAQLEADVKSAQSCSLDMYLRHHTCISGHAKEDELLDAVRVAPDVRREIMEKRSEVRQGWCERISKEAAAKCQTVIDDLTLMNGKQAQEITELRDSAEKYEKQIAELVSTITQNQITYQQELQALVAKNVELDALNQRQAKSLRITPSLLSATPIDSADGVADLIDFSVPTDEL

SEQ ID NO: 20 - protein, 204 aa, synthetic construct
  source 1..204: note = mammalian muNS-Mi N113S
VALQPLLSQLRELSSEVTRLQMELSRAQSLNAQLEADVKSAQSCSLDMYLRHHTCINGHAKEDELLDAVRVAPDVRREIMEKRSEVRQGWCERISKEAAAKCQTVIDDLTLMSGKQAQEITELRDSAEKYEKQIAELVSTITQNQITYQQELQALVAKNVELDALNQRQAKSLRITPSLLSATPIDSADGVADLIDFSVPTDEL

SEQ ID NO: 21 - protein, 204 aa, synthetic construct
  source 1..204: note = mammalian muNS-Mi N57S N113S
VALQPLLSQLRELSSEVTRLQMELSRAQSLNAQLEADVKSAQSCSLDMYLRHHTCISGHAKEDELLDAVRVAPDVRREIMEKRSEVRQGWCERISKEAAAKCQTVIDDLTLMSGKQAQEITELRDSAEKYEKQIAELVSTITQNQITYQQELQALVAKNVELDALNQRQAKSLRITPSLLSATPIDSADGVADLIDFSVPTDEL

SEQ ID NO: 22 - protein, 5 aa, synthetic construct
  source 1..5: note = Sortase recognition motif
LPXTG

SEQ ID NO: 23 - protein, 5 aa, synthetic construct
  source 1..5: note = Sortase recognition motif
LPETG

SEQ ID NO: 24 - skipped

SEQ ID NO: 25 - protein, 66 aa, Avian orthoreovirus
EDHLLAYLNEHVCVNAKDHEKGLLARCNVSGDSISSILGQRMKNRERFETRLRHEASAEWEPRVEA

SEQ ID NO: 26 - protein, 62 aa, Mammalian orthoreovirus
CSLDMYLRHHTCINGHAKEDELLDAVRVAPDVRREIMEKRSEVRQGWCERISKEAAAKCQTV

SEQ ID NO: 27 - DNA, 29 bp, synthetic construct
  source 1..29: mol_type = other DNA; note = positive primer
catgccatggcaccagccgtactgctgtc

SEQ ID NO: 28 - DNA, 43 bp, synthetic construct
  source 1..43: mol_type = other DNA; note = negative primer
ttgcggccgcaatcagccggtttccggcagcagatcatccacc

SEQ ID NO: 29 - protein, 5 aa, synthetic construct
GGGGS

SEQ ID NO: 30 - protein, 14 aa, synthetic construct
SGGTSGSTSGTGST

SEQ ID NO: 31 - protein, 15 aa, synthetic construct
AGSSTGSSTGPGSTT

SEQ ID NO: 32 - protein, 7 aa, synthetic construct
GGSGGAP

SEQ ID NO: 33 - protein, 8 aa, synthetic construct
GGGVEGGG

SEQ ID NO: 34 - protein, 10 aa, synthetic construct
PKPSTPPGSS

SEQ ID NO: 35 - protein, 5 aa, synthetic construct
AAALE

SEQ ID NO: 36 - DNA, 29 bp, synthetic construct
  source 1..29: mol_type = other DNA
catgccatggcaccagccgtactgctgtc

SEQ ID NO: 37 - DNA, 59 bp, synthetic construct
  source 1..59: mol_type = other DNA
ttgcggccgcaatcaaccaccagtctccgggcagagaaccaccacccagatcatccacc